European Patent Application EP 4 309 663 A1, published January 24, 2024. Title: MICROORGANISMS SYNTHESIZING ANTI-INFLAMMATORY MOLECULES. Applicant: Enbiosis Biotechnology Limited. The sequence listing filed with the application follows.

SEQUENCE LISTING (26 sequences)

SEQ ID NO: 1 - DNA, 408 bp, synthetic construct
  source 1..408: mol_type = other DNA
atgatgatgcctgcaaactactctgttatcgcagagaacgaaatgacctacgtcaacggtggcgctaacttcatcgacgctatcggcgctgttaccgctcctatctggactctggacaacgttaagaccttcaacaccaacatcgtgactctggttggcaacaccttcctgcagtccaccattaaccgcaccatcggtgtcctgttcagcggcaacaccacctggaaggaagtcggcaacatcggcaagaacctgttcggcaccaatgttaagggcaacccgatcgagaagaacaactttggtgactatgctatgaacgctctgggcattgctgctgctgtctacaacctgggcgtggctcccaccaagaacaccgtcaaggagactgaggttaagttcactgtctaa

SEQ ID NO: 2 - protein, 135 aa, synthetic construct
MMMPANYSVIAENEMTYVNGGANFIDAIGAVTAPIWTLDNVKTFNTNIVTLVGNTFLQSTINRTIGVLFSGNTTWKEVGNIGKNLFGTNVKGNPIEKNNFGDYAMNALGIAAAVYNLGVAPTKNTVKETEVKFTV

SEQ ID NO: 3 - DNA, 519 bp, synthetic construct
  source 1..519: mol_type = other DNA
atgtctgaacaacaggagtattggtttgccgctcggacaaagaaggaccaggagttttctgttcgcaatgctttagaaaagcttggaatagaatactttcttccaacacaatttgtcatccgtcaactgaaatatcgtcgtcgtagggtagaagttcctgttatcaagaatcttatttttgtccggaccacgaaagaccgtgcttggtctatcacgaaggatgatcatgttcctctttattatatgaaggatctctatacccatactttgttgatcgttcccaacaaacagatggaagatttcaagtttgtgatggatttagctccggaaaatgtaacttttgatgatcttccccttaccgttggtacaaaagtgcaggtcgtcaaaggagagttttgtggcattgagggcgaattgtccagccttgccaaccgtacttacgtagtgattcgtatccacggagttctttctgccagcgtcaaagtacctaaaagttaccttcgtattctttcagcgtaa

SEQ ID NO: 4 - protein, 172 aa, synthetic construct
MSEQQEYWFAARTKKDQEFSVRNALEKLGIEYFLPTQFVIRQLKYRRRRVEVPVIKNLIFVRTTKDRAWSITKDDHVPLYYMKDLYTHTLLIVPNKQMEDFKFVMDLAPENVTFDDLPLTVGTKVQVVKGEFCGIEGELSSLANRTYVVIRIHGVLSASVKVPKSYLRILSA

SEQ ID NO: 5 - DNA, 474 bp, synthetic construct
  source 1..474: mol_type = other DNA
atgaatcaagtccaaaatctgcaacacattgcccgtgagttgctttatttgggtatggatggttctcccatctataccgatcatttccgtcaactgaacaccgaagtttttcgcttgtccgaagcccttttctctatgaaaggtgccacatccgaggaagaagcagcgatttgtctgtccctgttaatgggctataatgctaccatttacaatgatggcgacaaagaatctaagatacaaagcattttagatcgctcttttgccgtattggaccatcttcccgcttctctattgaaatgccaattgctgacttattgctatggcgaggtattcgaggaggatttagcacaagaagcacatcaaataatggatagctggaaaaatagggcactttcagaagaagaattggaagtgatggagacattgcagacaatggaagataatcggtatccgtgtagcgaggtagaagattga

SEQ ID NO: 6 - protein, 157 aa, synthetic construct
MNQVQNLQHIARELLYLGMDGSPIYTDHFRQLNTEVFRLSEALFSMKGATSEEEAAICLSLLMGYNATIYNDGDKESKIQSILDRSFAVLDHLPASLLKCQLLTYCYGEVFEEDLAQEAHQIMDSWKNRALSEEELEVMETLQTMEDNRYPCSEVED

SEQ ID NO: 7 - DNA, 1449 bp, synthetic construct
  source 1..1449: mol_type = other DNA
atgggacaatcaataaagaataacttcctactgaatctaagtactacaattactgggctattatttccactaataacttttccctatgcttcacgtatattaatggcagatggtatagggcaagtacaatttttccaatccataattgactatgtctctctttgtactgctttgggaatccctttgtatgccgttagagaaattgcaagaataagggataataaggaattaagaagtagaacaacaatcgaaatactattgcttcatgctattttgactttagtcggatatatagttgtttttatacttgctaagaccgttgccaaaatagaaatagatgcttctcttttctttttgttaagtacaactttattttttaacacgataggagttgcatggttttatcaggcaattgaagattttaaatacataactttacgttccttatttgtaaggatactatctttagtggccttatttatctttgttaagaccaagcaagatctgttttattatgctggaatattagttattggtactgttggtaataatatatttaatttttttcgattacgtaaatatataaaacttagtaaaggcgaatttaagcgtttgaatctgttgaggcatttaatacctgcacttaaaatttttatattaaatttggttataagtatttatgtgaatcttgattctgtgatgcttggatttcttaaaaatgaagaatcagttggttattatgctgctgctactcgacttacaaaagctattttgggtatagtttcttcattaggagctgttttattacctcgttttagtaatatgataactaatggtcaaaaagaagaattccaattattggcaaataaagctgctagttttacaattgctttaagtcttcctatgagtgtgggacttatttttatggcagcacctattatacatattttttgtggaaatggttttgaaccttctattttgacattaaaattagttgcacctattgttttatttattggattatctggaattattggaatgcaaatattgtatccgcaagggagagaaaagtacgtaattatatctactatggtaggagcatgtataaatctccttataaactatttactaataccccaatatgggcagtatggagcggcgcttgggactgttatcgcagaatttatggtaacggttataatgattttgctgggaagaaaatatttacctataaatattctctccaagcagaatttacactatctaataggttctatagtgatatctattctattagcttttttgtttgtcttccctttacatgaagtaaattatttattgataggtatactgttatctgttattgtttattacgcatatttattaatgataaaagataccctcgcattacaactaaagaaattattactttcaatatttaaacaatga

SEQ ID NO: 8 - protein, 482 aa, synthetic construct
MGQSIKNNFLLNLSTTITGLLFPLITFPYASRILMADGIGQVQFFQSIIDYVSLCTALGIPLYAVREIARIRDNKELRSRTTIEILLLHAILTLVGYIVVFILAKTVAKIEIDASLFFLLSTTLFFNTIGVAWFYQAIEDFKYITLRSLFVRILSLVALFIFVKTKQDLFYYAGILVIGTVGNNIFNFFRLRKYIKLSKGEFKRLNLLRHLIPALKIFILNLVISIYVNLDSVMLGFLKNEESVGYYAAATRLTKAILGIVSSLGAVLLPRFSNMITNGQKEEFQLLANKAASFTIALSLPMSVGLIFMAAPIIHIFCGNGFEPSILTLKLVAPIVLFIGLSGIIGMQILYPQGREKYVIISTMVGACINLLINYLLIPQYGQYGAALGTVIAEFMVTVIMILLGRKYLPINILSKQNLHYLIGSIVISILLAFLFVFPLHEVNYLLIGILLSVIVYYAYLLMIKDTLALQLKKLLLSIFKQ

SEQ ID NO: 9 - DNA, 1095 bp, synthetic construct
  source 1..1095: mol_type = other DNA
atgaaaaaaaaatatgactatctaattgtcggagccggactttatggttctgtttttgcatataaagcgcaacggaatgggaaaaaatgtttgcttattgacaaacgtccacacaatggaggaaatatttattgcgaaaatattgagggtataaatgtacacaaatatggtgcacatatttttcatacttctaataaagaggtttgggactttgtaaatgccatagtggaatttaaccgctatactaattcccctattgccaattataaaggcaaattatataatttaccttttaatatgaatactttttatgctttatgggggacaaaaactccagaggaagcaaaaatgaagatagaagagcaaaggagagaagcggggattcttacgccgaagaatctagaagaacaggctatctctttagtaggaaaggatatttatgaaatattgataaaaggatatactgagaaacagtgggggcggaaagcaactgaacttcctgcttttataatcaagcgtttacctgtcagatttacttttgataataattactttaatgataaatatcaggggattcctgttggtggctataataaattgataaatggtttattagatggtattgaagttagaacaaatacagacttttttcaaaataaagaatattttaaaggtcttgcggataaaattctatttactggcaaaattgatgaatattataattatcaatttgggagattggaatatcgtactgttgaatttgaaacacaagtgcttgattgtgagaattatcaagggaatgcagttgtgaattatactgaaagggaagtgccttatactcgtattatagagcataaacattttgaatttggaacacagcccaaaaccgtaatttccaaagaatattcttcggaatggaaagatggtagtgaacccttttatcctgttaatgatgagaggaataattctttgtatttggagtataagaaattggtcgatagagagaagaatgttttgtttggagggagattagctgagtataagtattatgatatgaatgtgattgtggaaaaagttataaatagtgacttatga

SEQ ID NO: 10 - protein, 364 aa, synthetic construct
MKKKYDYLIVGAGLYGSVFAYKAQRNGKKCLLIDKRPHNGGNIYCENIEGINVHKYGAHIFHTSNKEVWDFVNAIVEFNRYTNSPIANYKGKLYNLPFNMNTFYALWGTKTPEEAKMKIEEQRREAGILTPKNLEEQAISLVGKDIYEILIKGYTEKQWGRKATELPAFIIKRLPVRFTFDNNYFNDKYQGIPVGGYNKLINGLLDGIEVRTNTDFFQNKEYFKGLADKILFTGKIDEYYNYQFGRLEYRTVEFETQVLDCENYQGNAVVNYTEREVPYTRIIEHKHFEFGTQPKTVISKEYSSEWKDGSEPFYPVNDERNNSLYLEYKKLVDREKNVLFGGRLAEYKYYDMNVIVEKVINSDL

SEQ ID NO: 11 - DNA, 876 bp, synthetic construct
  source 1..876: mol_type = other DNA
atgaagatatttgctgtagttgtgacctataatcgtttagcattactaaaaaaggtcatagatttacttaaaagacagacacgtcaattagatagtatagttatagtaaataatggctctactgatggaacaaaagaatggttagaacaggagaaaaatataacattaataaatcaatctaattctggtggggctggtggattcgaaacgggggtaaaatatgcatatgagaatgaggcagattggatttggatgatggatgatgatgtttttcctaatatagattgtttggaaaaactcttagggtggacgagtatttctcaatgtatccaaccacgtaggtattattcggatgatgtagaagtaaattttgaacaatggttggatccaattacttatagtaaatttggttattggcaagaaaaatcatttaataatggtaaaaagttttgtgctattaatgtaggctgttttgaagggatgtttgtttcgaaaagcattgttaataaaataggatttcctgataagcgtttttttatagcggaagatgatacaatatatgggtttgcagctagtttttataccaacgtaattttagtatctgatgctatcatggttcgtgctagaagatcatcggatcgtagcgttagcccaatgtatacttattatgcatgtcggaattttcatttagtatatgagtcacttaatttattattggataagaaaaataggtttttatatattaaatatatttatcaatttgttcatcagatttatttatctatttttttatatgataataagatgaaacacttaatatctgtttttcgtggcttttatgattgctttcgtaaaaaaaatggagctacctattaa

SEQ ID NO: 12 - protein, 291 aa, synthetic construct
MKIFAVVVTYNRLALLKKVIDLLKRQTRQLDSIVIVNNGSTDGTKEWLEQEKNITLINQSNSGGAGGFETGVKYAYENEADWIWMMDDDVFPNIDCLEKLLGWTSISQCIQPRRYYSDDVEVNFEQWLDPITYSKFGYWQEKSFNNGKKFCAINVGCFEGMFVSKSIVNKIGFPDKRFFIAEDDTIYGFAASFYTNVILVSDAIMVRARRSSDRSVSPMYTYYACRNFHLVYESLNLLLDKKNRFLYIKYIYQFVHQIYLSIFLYDNKMKHLISVFRGFYDCFRKKNGATY

SEQ ID NO: 13 - DNA, 1044 bp, synthetic construct
  source 1..1044: mol_type = other DNA
atgaggaagatattattaacatatggagatattaaaaccataaatattggtgattatattcagagtatcgccgctaaacaattttttgatgatgataattatatatttttcaatcgtgatgaattaaagttgtataaaggggaacctgcaaaagtcataatgaatgcttggatgacttataaaccatataattggcctccttcatctcaggtttatccattatttgttgcattacatatcaattcttctgcagaaagtcgctttttgtcacatgatagtattaagtatttaaaaaagtatgaacccatagggtgccgcgattatcatacaatgaatattttaaaaggaaaaggtgttaatgcttatttttcgggatgtcttactactactttgggtaaaacttataaatataatggaaaacgtgaggggatatacattgttgatccactttcatacatgcctaatgggaataatttttttgaaataatgaaagctgttgtacaaactgttttttatatgaagcctgtgctaaagattcttagaaattataaaaagaataatagatttactattaatatatccaaagtaggaataggacgtttattgttaataaccaagtcttatttgcttttgagaaagctagtagttcctgacgtattatacaatgcaatatttataacacaatttaatatgtctaatgaatattcttctgaatcagaaagatttgctcgggctgatgaattattaactaaaatggcctcagctcaatatgtgataacttctagaatccactgtgctcttccttgcttaggctttgagacccctgtggtttatattagaaatctatcagaaagcaagaagagcacttgtcgattagggggacttgaatctctatttaatgtgataactgtgaagggggaaaatgttacttccaatttttttgatggactatttaaacgagattcttcttttaagaataaaattgattttgtagaatatagagatcgattaattaatatatgtaataaatttatgatgtcatga

SEQ ID NO: 14 - protein, 347 aa, synthetic construct
MRKILLTYGDIKTINIGDYIQSIAAKQFFDDDNYIFFNRDELKLYKGEPAKVIMNAWMTYKPYNWPPSSQVYPLFVALHINSSAESRFLSHDSIKYLKKYEPIGCRDYHTMNILKGKGVNAYFSGCLTTTLGKTYKYNGKREGIYIVDPLSYMPNGNNFFEIMKAVVQTVFYMKPVLKILRNYKKNNRFTINISKVGIGRLLLITKSYLLLRKLVVPDVLYNAIFITQFNMSNEYSSESERFARADELLTKMASAQYVITSRIHCALPCLGFETPVVYIRNLSESKKSTCRLGGLESLFNVITVKGENVTSNFFDGLFKRDSSFKNKIDFVEYRDRLINICNKFMMS

SEQ ID NO: 15 - DNA, 1137 bp, synthetic construct
  source 1..1137: mol_type = other DNA
atgagggatggaaagcccattgaaatactgcatattgtagggactagacctgttggaggaattggtgctttattgaaaaatataaacacttctattgatttaaataaattccattttacatatgtgttttctgccgatagtaatattggagattttgataattatgtgagaaaattaggtagcgatattgttgtattcccttcatatcatttgaaatatttatttttatatttaaaggtgattttctgtttttataagagaaatgcaaaaaaatatgatataattcatgtacatagtgctaatacaggagtattagaccttttatttgcaaagatatatggaatacggataaggattttacatagtcacagtacaaaatattctagtaaaaaaataaggtccattagaaattattttttgcaatttcctacaatatatttagcaaacacttattttgcatgtggatacaaagctgctgaattcctttttggaaaaaagagacttgaaaaagtttatattattcataatgcaattttttctaaaaaatttatttataatgcaactgttagagagagagttagagttgagttgaaaatagagaatgactgtttactgttggggcatatcggtaactttacgaaagaaaagaatcatggttttttaatagatatattggaagaattattgaatattaatgacaatgttaagttgctgttagtaggggatggccaacttagaagtgaaatagaggaaaaagtaaaattaaaaagattgcagaagtatgtgtgctttttaggtcggagaactgatatatcagaattattacaagctatggattttttaatttttccttctttttttgaaggtctaccagtgactctgattgaagcgcaagcttctggtttaagatgtgtcgtttcggatcgtattactttggaaacaaagataacgaataatataagttatcttaatctcaatcgagatccttcaacttgggctgaagttgtttggaagttgtttgaagataaaacttttatcaggaaagatacgtctaaagaaatatgtgaatcaggatatgatatacatttagagagtgaatatctcgaaagaatatatttaaatcttttacataaatga

SEQ ID NO: 16 - protein, 378 aa, synthetic construct
MRDGKPIEILHIVGTRPVGGIGALLKNINTSIDLNKFHFTYVFSADSNIGDFDNYVRKLGSDIVVFPSYHLKYLFLYLKVIFCFYKRNAKKYDIIHVHSANTGVLDLLFAKIYGIRIRILHSHSTKYSSKKIRSIRNYFLQFPTIYLANTYFACGYKAAEFLFGKKRLEKVYIIHNAIFSKKFIYNATVRERVRVELKIENDCLLLGHIGNFTKEKNHGFLIDILEELLNINDNVKLLLVGDGQLRSEIEEKVKLKRLQKYVCFLGRRTDISELLQAMDFLIFPSFFEGLPVTLIEAQASGLRCVVSDRITLETKITNNISYLNLNRDPSTWAEVVWKLFEDKTFIRKDTSKEICESGYDIHLESEYLERIYLNLLHK

SEQ ID NO: 17 - DNA, 807 bp, synthetic construct
  source 1..807: mol_type = other DNA
atgaaattggctgtcatttcttctatctacaaaaatgattcgctttctaaaataaagcaatccttacaaagtttgttgaatcaagaaaatgttacttgtgatatttatttatattgtgatggtcctgtttcgattgatattgtgcatttcttagactcatttgatcaaaactcactttatatatttaagcaagaacaaaatagaggattggctcatgcactaaatgaattattgaatatcgttcttacaaaagaatacgaatatattgctcgtatggatgctgatgatatttccatgccggaacgttttgtgaagcagatcgcatttatgaattcacatccggatattgattgccttggtacttgggcaatagaaattgatgatgacggaaaagaatattttcgaaaaaaaatgccgataactcatgaagaatgtttggaactgtttaaaaagcgggattgtatgattcatcctactgtgatgtttcgacgttcatattttgagaaagctggtttatatcccgaagacacctactttggagaagatactatgatgtgggctaaaggttttaaaagtggatgtaaatttgccaatgtacccgaatatctgtttaagtttagattggattcaaacttctttgaaagaaggcgggggtggaaacatgcaaaatctatttatactttacgtcatcgtgttaatagaatgttagggttcggatggaaggaagattgttatgcattgctatatgctatggccaaattaatgcctaaatctattcttgacataatctataaaacagtacgttga

SEQ ID NO: 18 - protein, 268 aa, synthetic construct
MKLAVISSIYKNDSLSKIKQSLQSLLNQENVTCDIYLYCDGPVSIDIVHFLDSFDQNSLYIFKQEQNRGLAHALNELLNIVLTKEYEYIARMDADDISMPERFVKQIAFMNSHPDIDCLGTWAIEIDDDGKEYFRKKMPITHEECLELFKKRDCMIHPTVMFRRSYFEKAGLYPEDTYFGEDTMMWAKGFKSGCKFANVPEYLFKFRLDSNFFERRRGWKHAKSIYTLRHRVNRMLGFGWKEDCYALLYAMAKLMPKSILDIIYKTVR

SEQ ID NO: 19 - DNA, 1224 bp, synthetic construct
  source 1..1224: mol_type = other DNA
atgaaaatacctttttcaccaccttatattgacgaggcggtcatcaacgaagtcgttgattcgttacgttccggttggatcacatccggtccgaaagtgaaggctttggaggaagaaattaaatctttctcaggagcaaaagaagtgctttgtgtcaattcctggacatcaggagctattatgatgttgcgttggctgggagtgaaggagggcgatgaagtgattgttcctgcctatacttacagtgcaacggcattggctgtgctccatgccggagccaaaccggtaatggtggattccggaactgattttaatatttcggtggaggctgttcgtaaagctattactcctaaaacaaaggcgattatacccgtagatattgctggttttccctgcgattatgaaagaatcatggcactggtgcaggaaccagaaatggtaaaactgttccgttcggaatctcctgtgcaagaaaaattgggacgcatcttggtgatgaatgatgctgcccactctttgggagcacgttacagtagccgtcagcgtaccggttgtgaaactgatgtggctatcttttcacttcatgccgtgaaaaatgtgactactgccgaaggtggggccatttgcctgaatctgcctaagccgttcgataatacggagttgtataaagagctacggatgacaagcttgaactgccagaccaaggatgctttttcgaaatctaaagccggaggatggcgttatgatattgtcggtttcgggatgaaaatcaatatggccgatgtaaatgccgccataggactggcacagatacgagaatatccggaattgctgaaagaacgaaagcgggtgtttaatgcttatagcgatgctttttcggcttgtgactgggccatcgttccgccttctgtggatggggaaaaggaaagctcttatcacatttatgctttgcgtattaaggactttaccgaagaacaacgcgaccggatgattgatgaaatcgctaaaagtgaagtggctgtcaatgtgcactttataccgatgccgatgttgtcgttcttcaaatcgatgggatatgatataaaggattatccacaggcttatcagaactttaagagcgagatatcattgccgatatatccccaattggatagtgaaaaattgaatttcattattgaaaccgtaaaggcggcctatgcgaccgtaattgcagaaaaccgatag

SEQ ID NO: 20 - protein, 407 aa, synthetic construct
MKIPFSPPYIDEAVINEVVDSLRSGWITSGPKVKALEEEIKSFSGAKEVLCVNSWTSGAIMMLRWLGVKEGDEVIVPAYTYSATALAVLHAGAKPVMVDSGTDFNISVEAVRKAITPKTKAIIPVDIAGFPCDYERIMALVQEPEMVKLFRSESPVQEKLGRILVMNDAAHSLGARYSSRQRTGCETDVAIFSLHAVKNVTTAEGGAICLNLPKPFDNTELYKELRMTSLNCQTKDAFSKSKAGGWRYDIVGFGMKINMADVNAAIGLAQIREYPELLKERKRVFNAYSDAFSACDWAIVPPSVDGEKESSYHIYALRIKDFTEEQRDRMIDEIAKSEVAVNVHFIPMPMLSFFKSMGYDIKDYPQAYQNFKSEISLPIYPQLDSEKLNFIIETVKAAYATVIAENR

SEQ ID NO: 21 - DNA, 597 bp, synthetic construct
  source 1..597: mol_type = other DNA
ataagttgcttgatccgtttttttgatatcgttttttcccttttgggaattcttctgctttctcccgtttttcttcttctttatatagccatttgtctcgaaagtaaaggaggtggtttctataaacagctccgtgtgggaaggtacggaggggatttttatgtttataaatttcgttcgatgcgtgtaggggctgataaaaaggggttgataacggtaggagggagagatccgagaataactcgtaccggatacctgatccggaagtataaattggatgaattgcctcagttgtttaacgtactgaaaggagatatgagtctggtagggccccgtcctgaggttcgtaagtatgtggatttatataccgatgaacaaaagaaagtattgagtgtacgtccggggattacggattatgcttctattgagtatgtagatgaaaatatgattcttggagaggcttcggatcctgacagagcatatatagaacagattatgcccgataagatacggtataatatgaaatatatctgtaatcgttcggtgaaggaatattttaaaattatatttctgacattttggagcatcattcgttag

SEQ ID NO: 22 - protein, 258 aa, synthetic construct
MFDKNKVKLGIAPIAWTNDDLPDLGAENTFEQCVSEMALAGFTGSEVGNKYPKDPAELKKMSCLIRFFDIVFSLLGILLLSPVFLLLYIAICLESKGGGFYKQLRVGRYGGDFYVYKFRSMRVGADKKGLITVGGRDPRITRTGYLIRKYKLDELPQLFNVLKGDMSLVGPRPEVRKYVDLYTDEQKKVLSVRPGITDYASIEYVDENMILGEASDPDRAYIEQIMPDKIRYNMKYICNRSVKEYFKIIFLTFWSIIR

SEQ ID NO: 23 - DNA, 597 bp, synthetic construct
  source 1..597: mol_type = other DNA
atgaagaaaaactttttttatgcaggtggtctgtcattgcttctttggggtatggcagcatgttccggacaaggaaaagcggataaagcagctgttgttgcggatagtgtagtggtgaaaacggatagtgttgcggcagacagcacaggatatattgtgaaagtgggagagtcagctcccgattttaccattactctgaccgacggaaagcagatgaaactctccgaacttcgcggtaaagtggtgatgttgcagttcacagccagctggtgcggagtatgccgtaaagagatgccttttatagagaaagatatctggctgaagcataaaaacaatcctgagtttgctttgataggcattgaccgtgacgaacctctcgataaggtgatcgcatttggaaagtcggtaggggtgacgtatccgttgggattggatccgggagcggatatctttgcgaagtatgcattgcgtgaatcgggcatcacccggaatgtcctgatagaccgggagggtaagattgtgaagctgactcgtttatataacgaagaggagtttgcctcactggtggatcaaatagatgaaatgctgaaaaaataa

SEQ ID NO: 24 - protein, 198 aa, synthetic construct
MKKNFFYAGGLSLLLWGMAACSGQGKADKAAVVADSVVVKTDSVAADSTGYIVKVGESAPDFTITLTDGKQMKLSELRGKVVMLQFTASWCGVCRKEMPFIEKDIWLKHKNNPEFALIGIDRDEPLDKVIAFGKSVGVTYPLGLDPGADIFAKYALRESGITRNVLIDREGKIVKLTRLYNEEEFASLVDQIDEMLKK

SEQ ID NO: 25 - DNA, 778 bp, synthetic construct
  source 1..778: mol_type = other DNA
ttataaggcaacagtcagccgggccagatagtcatagtgcttaccctcttttatcatttcggccttgaagccattgtcggcagcataggcgctgagggtctggaagtcgatatacagccagtcgaaaggatcgccttgaatatctttatattgcatgcggaagtcaatttctccataataatctcctgccaggtcgatcaggaagctgccgtcttcatcttcgaacagatagcggaggtcactcgaatccatcaggatgcaaccatccgggcggagtaattgtttcatcttgcggaagaagagaggcatattctccaaacgtccgataatgccggaaccgttcatcaacataaggatggtatcgaaagtcgcggcaaagcgttcgtcgaacagattgacttggcgggcatctttcactccccgcagtttcatcacttcgacggataaaggggagatgtcgatggcggaaacttctttaccgctctcttgaagggcaagagcgtggcaaccgcttccggcacctacgtcgagtattgttccggtagccattgcgagggctgtgcgttcgagtagaggcatttgtccggctttgcggaaaagttgtttgacgggtatttcgtcttcatcgaactgagaagaaaatacgcgtaatctgtctgctttttggcgatgataaaaatcggctatggcagcacccatggggtctttttctgccgggagcagggatgtattcattgattggtttttagttgttacagcgggcaaagatagggaattc

SEQ ID NO: 26 - protein, 258 aa, synthetic construct
NSLSLPAVTTKNQSMNTSLLPAEKDPMGAAIADFYHRQKADRLRVFSSQFDEDEIPVKQLFRKAGQMPLLERTALAMATGTILDVGAGSGCHALALQESGKEVSAIDISPLSVEVMKLRGVKDARQVNLFDERFAATFDTILMLMNGSGIIGRLENMPLFFRKMKQLLRPDGCILMDSSDLRYLFEDEDGSFLIDLAGDYYGEIDFRMQYKDIQGDPFDWLYIDFQTLSAYAADNGFKAEMIKEGKHYDYLARLTVAL